European Patent Specification EP 3 556 863 B1, published September 18, 2024. Title: ASSAYS FOR IGFBP7 HAVING IMPROVED PERFORMANCE IN BIOLOGICAL SAMPLES. Applicant: ASTUTE MEDICAL, INC. Application PCT/US2014/064327. The sequence listing filed with the application follows.

SEQUENCE LISTING (12 sequences)

SEQ ID NO: 1 - protein, 26 aa, Homo sapiens
LIWNKVKRGHYGVQRTELLPGDRDNL

SEQ ID NO: 2 - protein, 20 aa, Homo sapiens
SSSSSDTCGPCEPASCPPLP

SEQ ID NO: 3 - protein, 9 aa, Homo sapiens
TELLPGDRD

SEQ ID NO: 4 - protein, 5 aa, Homo sapiens
EPASC

SEQ ID NO: 5 - protein, 282 aa, Homo sapiens
MERPSLRALLLGAAGLLLLLLPLSSSSSSDTCGPCEPASCPPLPPLGCLLGETRDACGCCPMCARGEGEPCGGGGAGRGYCAPGMECVKSRKRRKGKAGAAAGGPGVSGVCVCKSRYPVCGSDGTTYPSGCQLRAASQRAESRGEKAITQVSKGTCEQGPSIVTPPKDIWNVTGAQVYLSCEVIGIPTPVLIWNKVKRGHYGVQRTELLPGDRDNLAIQTRGGPEKHEVTGWVLVSPLSKEDAGEYECHASNSQGQASASAKITVVDALHEIPVKKGEGAEL

SEQ ID NO: 6 - protein, 16 aa, Homo sapiens
YGVQRTELLPGDRDNL

SEQ ID NO: 7 - protein, 16 aa, Homo sapiens
LIWNKVKRGHYGVQRT

SEQ ID NO: 8 - protein, 20 aa, Homo sapiens
SSSSSDTCGPCEPASCPPLP

SEQ ID NO: 9 - protein, 110 aa, Artificial Sequence
  Description of Artificial Sequence: Synthetic polypeptide
DVVMTQTPLTLSVTIGQPASISCKSSQSLLYSNGETYLHWLLQRPGQSPKRLIYLVSKLDSGVPDRFTGSGSRTDFTLKISRVEAEDLGVYYCAQGTHFPHTFGGGTKLE

SEQ ID NO: 10 - protein, 111 aa, Artificial Sequence
  Description of Artificial Sequence: Synthetic polypeptide
QIQLVQSGPELKKPGETVKISCKASGYSFTDYSIHWVKQAPGKGLKWMGLINTETGEPIYVDDFKGRFAFSLETSARTAYLQINNLKNEDTATYFCARAYYWAYWGQGTLV

SEQ ID NO: 11 - protein, 107 aa, Artificial Sequence
  Description of Artificial Sequence: Synthetic polypeptide
QIVLTQSPAIMSASPGEKVTMTCSASSSVSYMHWYQQKSGTSPKRWIYDTSELASGVPARFSGSGSGTSYSLTISSMEAEDAATYYCQQWSSSPFTFGSGTKLEIKR

SEQ ID NO: 12 - protein, 120 aa, Artificial Sequence
  Description of Artificial Sequence: Synthetic polypeptide
QIQLVQSGPELKKPGETVKISCKASGYTFKKYGMNWVKQAPGKGLKWMGWINTYTGEPIYADDFKGRFAFSLETSASTAYLQISNLKNEDTATYFCAREEYGPFYAMDYWGQGTSVTVSS